European Patent Application EP 4 567 108 A1, published June 11, 2025. Title: Screening of target peptides using fusion polypeptides. Applicant: Christoph Kutzner. Application EP. The sequence listing filed with the application follows.

SEQUENCE LISTING (14 sequences)

SEQ ID NO: 1 - protein, 268 aa, synthetic construct
VYVKPVYVKVYVPNIHYWNTTGTTTGTTWPTAMKEEGEEIYSIIIPSSSGDVSIIIPNIHYWNTTGTTTWPTAMKEIYSIIIPSSSGDVSIIIPNIHYWNTTGTTWPAMKEDGEIYSIIIPSGDVSIIINDGNNVYVKPVYVKVYVPNIHYWNTTGTTTGTTWPTAMKEEGEEIYSIIIPSSSGDVSIIIPNIHYWNTTGTTTWPTAMKEIYSIIIPSSSGDVSIIIPNIHYWNTTGTTWPAMKEDGEIYSIIIPSGDVSIIINDGNN

SEQ ID NO: 2 - protein, 142 aa, synthetic construct
GVEEYCYNISGRPVIGDPTEVYPDNISKVPHDKGRGNIGTSIRNLPRRGNCRVCYSGQYIGIYGPVFYQDVANAELPRMLVEHKTKICHVVKRIGRVTGSLYHVLKCINGCNVIKYSRCGLEPSSLKWIRNFTDCPLWVTSC

SEQ ID NO: 3 - protein, 150 aa, synthetic construct
GVEEPVYDATGKPLFGDPSEVHPQTLLKLPHDRGRGNIKTTLKDLPRKGDCDSGNRLGPVSGIYVKPGPVFYQDFMGPLYHRAPLEYYSEAKQIQVTLLIGRVTSSDGDAGGILLCIHGVIGLVLAGGGEPVTFKDLRNFTDCPLWVTSC

SEQ ID NO: 4 - protein, 25 aa, synthetic construct
MAVLKTRRSTRRSTRRAVLKDWEAM

SEQ ID NO: 5 - protein, 43 aa, synthetic construct
EGSKESGSVSSEQLAQFRSLDAGSASELNHFELLYKTNKQKPV

SEQ ID NO: 6 - protein, 478 aa, synthetic construct
MAVLKTRRSTRRSTRRAVLKDWEAMVYVKPVYVKVYVPNIHYWNTTGTTTGTTWPTAMKEEGEEIYSIIIPSSSGDVSIIIPNIHYWNTTGTTTWPTAMKEIYSIIIPSSSGDVSIIIPNIHYWNTTGTTWPAMKEDGEIYSIIIPSGDVSIIINDGNNVYVKPVYVKVYVPNIHYWNTTGTTTGTTWPTAMKEEGEEIYSIIIPSSSGDVSIIIPNIHYWNTTGTTTWPTAMKEIYSIIIPSSSGDVSIIIPNIHYWNTTGTTWPAMKEDGEIYSIIIPSGDVSIIINDGNNEGSKESGSVSSEQLAQFRSLDAGSASELNHFELLYKTNKQKPVGVEEYCYNISGRPVIGDPTEVYPDNISKVPHDKGRGNIGTSIRNLPRRGNCRVCYSGQYIGIYGPVFYQDVANAELPRMLVEHKTKICHVVKRIGRVTGSLYHVLKCINGCNVIKYSRCGLEPSSLKWIRNFTDCPLWVTSC

SEQ ID NO: 7 - protein, 486 aa, synthetic construct
MAVLKTRRSTRRSTRRAVLKDWEAMVYVKPVYVKVYVPNIHYWNTTGTTTGTTWPTAMKEEGEEIYSIIIPSSSGDVSIIIPNIHYWNTTGTTTWPTAMKEIYSIIIPSSSGDVSIIIPNIHYWNTTGTTWPAMKEDGEIYSIIIPSGDVSIIINDGNNVYVKPVYVKVYVPNIHYWNTTGTTTGTTWPTAMKEEGEEIYSIIIPSSSGDVSIIIPNIHYWNTTGTTTWPTAMKEIYSIIIPSSSGDVSIIIPNIHYWNTTGTTWPAMKEDGEIYSIIIPSGDVSIIINDGNNEGSKESGSVSSEQLAQFRSLDAGSASELNHFELLYKTNKQKPVGVEEPVYDATGKPLFGDPSEVHPQTLLKLPHDRGRGNIKTTLKDLPRKGDCDSGNRLGPVSGIYVKPGPVFYQDFMGPLYHRAPLEYYSEAKQIQVTLLIGRVTSSDGDAGGILLCIHGVIGLVLAGGGEPVTFKDLRNFTDCPLWVTSC

SEQ ID NO: 8 - DNA, 804 bp, synthetic construct
  source 1..804: mol_type = other DNA
gtgtatgtgaaaccggtgtatgtgaaagtgtatgtgccgaacattcattattggaacaccaccggcaccaccaccggcaccacctggccgaccgcgatgaaagaagaaggcgaagaaatttatagcattattattccgagcagcagcggcgatgtgagcattattattccgaacattcattattggaacaccaccggcaccaccacctggccgaccgcgatgaaagaaatttatagcattattattccgagcagcagcggcgatgtgagcattattattccgaacattcattattggaacaccaccggcaccacctggccggcgatgaaagaagatggcgaaatttatagcattattattccgagcggcgatgtgagcattattattaacgatggcaacaacgtgtatgtgaaaccggtgtatgtgaaagtgtatgtgccgaacattcattattggaacaccaccggcaccaccaccggcaccacctggccgaccgcgatgaaagaagaaggcgaagaaatttatagcattattattccgagcagcagcggcgatgtgagcattattattccgaacattcattattggaacaccaccggcaccaccacctggccgaccgcgatgaaagaaatttatagcattattattccgagcagcagcggcgatgtgagcattattattccgaacattcattattggaacaccaccggcaccacctggccggcgatgaaagaagatggcgaaatttatagcattattattccgagcggcgatgtgagcattattattaacgatggcaacaac

SEQ ID NO: 9 - DNA, 426 bp, synthetic construct
  source 1..426: mol_type = other DNA
ggcgccgaagaatattgctataacattagcggccgcccggtgattggcgatccgaccgaagtgtatccggataacattagcaaagtgccgcatgataaaggccgcggcaacattggcaccagcattcgcaacctgccgcgccgcggcaactgccgcgtgtgctatagcggccagtatattggcatttatggcccggtgttttatcaggatgtggcgaacgcggaactgccgcgcatgctggtggaacataaaaccaaaatttgccatgtggtgaaacgcattggccgcgtgaccggcagcctgtatcatgtgctgaaatgcattaacggctgcaacgtgattaaatatagccgctgcggcctggaaccgagcagcctgaaatggattcgcaactttaccgattgcccgctgtgggtgaccagctgc

SEQ ID NO: 10 - DNA, 446 bp, synthetic construct
  source 1..446: mol_type = other DNA
ggcgtggaagaacatgtgtatgatgcgaccggcaaactgtttggcgatccgagcgaagtgcatccgcagaccctgctgaaactgccgcatgatcgcggccgcggcaacattaaaaccaccctgaaagatctgccgcgcaaaggcgattgcgatagcggcaaccgcctgggcccggtgagcggcatttatgtgaaaccgggcccggtgttttatcaggattttatgggcccgctgtatcatcgcgcgccgctggaatattatagcgatgcgaaacagattcaggtgaccctgctgattggccgcgtgaccagcagcgatggcgatgcgggcggcattctgctgtgcattcatggcgtgattggcctggtgctggcgggcggcggcgaaccggtgacctttaaagatctgcgcaactttaccgattgccgctgtgggtgaccagctgc

SEQ ID NO: 11 - DNA, 78 bp, synthetic construct
  source 1..78: mol_type = other DNA
catatggcggtgctgaaaacccgccgcagcacccgccgcagcacccgccgcgcggtgctgaaagattgggaacatatg

SEQ ID NO: 12 - DNA, 132 bp, synthetic construct
  source 1..132: mol_type = other DNA
ggaggcaaagaaagcggcagcgtgagcagcgaacagctggcgcagtttcgcagcctggatgcgggcagcgcgagcgaactgaaccattttgaactgctgtataaaaccaacaaacagaaaccggtgggcgcc

SEQ ID NO: 13 - DNA, 1434 bp, synthetic construct
  source 1..1434: mol_type = other DNA
catatggcggtgctgaaaacccgccgcagcacccgccgcagcacccgccgcgcggtgctgaaagattgggaacatatggtgtatgtgaaaccggtgtatgtgaaagtgtatgtgccgaacattcattattggaacaccaccggcaccaccaccggcaccacctggccgaccgcgatgaaagaagaaggcgaagaaatttatagcattattattccgagcagcagcggcgatgtgagcattattattccgaacattcattattggaacaccaccggcaccaccacctggccgaccgcgatgaaagaaatttatagcattattattccgagcagcagcggcgatgtgagcattattattccgaacattcattattggaacaccaccggcaccacctggccggcgatgaaagaagatggcgaaatttatagcattattattccgagcggcgatgtgagcattattattaacgatggcaacaacgtgtatgtgaaaccggtgtatgtgaaagtgtatgtgccgaacattcattattggaacaccaccggcaccaccaccggcaccacctggccgaccgcgatgaaagaagaaggcgaagaaatttatagcattattattccgagcagcagcggcgatgtgagcattattattccgaacattcattattggaacaccaccggcaccaccacctggccgaccgcgatgaaagaaatttatagcattattattccgagcagcagcggcgatgtgagcattattattccgaacattcattattggaacaccaccggcaccacctggccggcgatgaaagaagatggcgaaatttatagcattattattccgagcggcgatgtgagcattattattaacgatggcaacaacggaggcaaagaaagcggcagcgtgagcagcgaacagctggcgcagtttcgcagcctggatgcgggcagcgcgagcgaactgaaccattttgaactgctgtataaaaccaacaaacagaaaccggtgggcgccgaagaatattgctataacattagcggccgcccggtgattggcgatccgaccgaagtgtatccggataacattagcaaagtgccgcatgataaaggccgcggcaacattggcaccagcattcgcaacctgccgcgccgcggcaactgccgcgtgtgctatagcggccagtatattggcatttatggcccggtgttttatcaggatgtggcgaacgcggaactgccgcgcatgctggtggaacataaaaccaaaatttgccatgtggtgaaacgcattggccgcgtgaccggcagcctgtatcatgtgctgaaatgcattaacggctgcaacgtgattaaatatagccgctgcggcctggaaccgagcagcctgaaatggattcgcaactttaccgattgcccgctgtgggtgaccagctgc

SEQ ID NO: 14 - DNA, 1454 bp, synthetic construct
  source 1..1454: mol_type = other DNA
catatggcggtgctgaaaacccgccgcagcacccgccgcagcacccgccgcgcggtgctgaaagattgggaacatatggtgtatgtgaaaccggtgtatgtgaaagtgtatgtgccgaacattcattattggaacaccaccggcaccaccaccggcaccacctggccgaccgcgatgaaagaagaaggcgaagaaatttatagcattattattccgagcagcagcggcgatgtgagcattattattccgaacattcattattggaacaccaccggcaccaccacctggccgaccgcgatgaaagaaatttatagcattattattccgagcagcagcggcgatgtgagcattattattccgaacattcattattggaacaccaccggcaccacctggccggcgatgaaagaagatggcgaaatttatagcattattattccgagcggcgatgtgagcattattattaacgatggcaacaacgtgtatgtgaaaccggtgtatgtgaaagtgtatgtgccgaacattcattattggaacaccaccggcaccaccaccggcaccacctggccgaccgcgatgaaagaagaaggcgaagaaatttatagcattattattccgagcagcagcggcgatgtgagcattattattccgaacattcattattggaacaccaccggcaccaccacctggccgaccgcgatgaaagaaatttatagcattattattccgagcagcagcggcgatgtgagcattattattccgaacattcattattggaacaccaccggcaccacctggccggcgatgaaagaagatggcgaaatttatagcattattattccgagcggcgatgtgagcattattattaacgatggcaacaacggaggcaaagaaagcggcagcgtgagcagcgaacagctggcgcagtttcgcagcctggatgcgggcagcgcgagcgaactgaaccattttgaactgctgtataaaaccaacaaacagaaaccggtgggcgtggaagaacatgtgtatgatgcgaccggcaaactgtttggcgatccgagcgaagtgcatccgcagaccctgctgaaactgccgcatgatcgcggccgcggcaacattaaaaccaccctgaaagatctgccgcgcaaaggcgattgcgatagcggcaaccgcctgggcccggtgagcggcatttatgtgaaaccgggcccggtgttttatcaggattttatgggcccgctgtatcatcgcgcgccgctggaatattatagcgatgcgaaacagattcaggtgaccctgctgattggccgcgtgaccagcagcgatggcgatgcgggcggcattctgctgtgcattcatggcgtgattggcctggtgctggcgggcggcggcgaaccggtgacctttaaagatctgcgcaactttaccgattgccgctgtgggtgaccagctgc